European Patent Specification EP 3 322 824 B1, published March 4, 2026. Title: DETECTION OF TUMOR-DERIVED DNA IN CEREBROSPINAL FLUID. Applicant: The Johns Hopkins University. The sequence listing filed with the application follows.

SEQUENCE LISTING (70 sequences)

SEQ ID NO: 1 - DNA, 46 bp, Artificial Sequence
  Synthetic primers
cacacaggaaacagctatgaccatgcttcaggtggctcgagtagtg

SEQ ID NO: 2 - DNA, 45 bp, Artificial Sequence
  Synthetic primers
cacacaggaaacagctatgaccatgtttcttttgcctgcaggatt

SEQ ID NO: 3 - DNA, 48 bp, Artificial Sequence
  Synthetic primers
cacacaggaaacagctatgaccatgtggacaatgtggagataaaggac

SEQ ID NO: 4 - DNA, 43 bp, Artificial Sequence
  Synthetic primers
cacacaggaaacagctatgaccatgctggtcctgcctcactcg

SEQ ID NO: 5 - DNA, 45 bp, Artificial Sequence
  Synthetic primers
cacacaggaaacagctatgaccatggaagcaaacagctcgcaagt

SEQ ID NO: 6 - DNA, 44 bp, Artificial Sequence
  Synthetic primers
cacacaggaaacagctatgaccatggccagctgttgctgaccta

SEQ ID NO: 7 - DNA, 45 bp, Artificial Sequence
  Synthetic primers
cacacaggaaacagctatgaccatgagacctcaggcggctcatag

SEQ ID NO: 8 - DNA, 45 bp, Artificial Sequence
  Synthetic primers
cacacaggaaacagctatgaccatggagtggttggggaggacatt

SEQ ID NO: 9 - DNA, 43 bp, Artificial Sequence
  Synthetic primers
cacacaggaaacagctatgaccatgctgtcaaggcgggcttct

SEQ ID NO: 10 - DNA, 45 bp, Artificial Sequence
  Synthetic primers
cacacaggaaacagctatgaccatgatcgggcagtgatagagcag

SEQ ID NO: 11 - DNA, 45 bp, Artificial Sequence
  Synthetic primers
cacacaggaaacagctatgaccatggaagcctctgattggcacag

SEQ ID NO: 12 - DNA, 55 bp, Artificial Sequence
  Synthetic primers
cacacaggaaacagctatgaccatggcttgtgagtggatgggtaaaacctatcat

SEQ ID NO: 13 - DNA, 55 bp, Artificial Sequence; identical to SEQ ID NO: 12
  Synthetic primers

SEQ ID NO: 14 - DNA, 53 bp, Artificial Sequence
  Synthetic primers
cacacaggaaacagctatgaccatgtccactacaactacatgtgtaacagttc

SEQ ID NO: 15 - DNA, 42 bp, Artificial Sequence
  Synthetic primers
cacacaggaaacagctatgaccatggcggaaaggaaggggag

SEQ ID NO: 16 - DNA, 42 bp, Artificial Sequence; identical to SEQ ID NO: 15
  Synthetic primers

SEQ ID NO: 17 - DNA, 47 bp, Artificial Sequence
  Synthetic primers
cacacaggaaacagctatgaccatgtggctctgactgtaccaccatc

SEQ ID NO: 18 - DNA, 44 bp, Artificial Sequence
  Synthetic primers
cacacaggaaacagctatgaccatgcggaaatgtgggaggagag

SEQ ID NO: 19 - DNA, 45 bp, Artificial Sequence
  Synthetic primers
cacacaggaaacagctatgaccatgccagcacctatggcaagttt

SEQ ID NO: 20 - DNA, 47 bp, Artificial Sequence
  Synthetic primers
cacacaggaaacagctatgaccatggccctgactttcaactctgtct

SEQ ID NO: 21 - DNA, 45 bp, Artificial Sequence
  Synthetic primers
cacacaggaaacagctatgaccatggtccaacgtgccatatccat

SEQ ID NO: 22 - DNA, 44 bp, Artificial Sequence
  Synthetic primers
cacacaggaaacagctatgaccatgccttgtggcaccctaggtc

SEQ ID NO: 23 - DNA, 44 bp, Artificial Sequence
  Synthetic primers
cacacaggaaacagctatgaccatgggaagttgatccgctcaca

SEQ ID NO: 24 - DNA, 42 bp, Artificial Sequence; identical to SEQ ID NO: 15
  Synthetic primers

SEQ ID NO: 25 - DNA, 42 bp, Artificial Sequence; identical to SEQ ID NO: 15
  Synthetic primers

SEQ ID NO: 26 - DNA, 42 bp, Artificial Sequence; identical to SEQ ID NO: 15
  Synthetic primers

SEQ ID NO: 27 - DNA, 42 bp, Artificial Sequence; identical to SEQ ID NO: 15
  Synthetic primers

SEQ ID NO: 28 - DNA, 48 bp, Artificial Sequence
  Synthetic primers
cacacaggaaacagctatgaccatggcaattcactgtaaagctggaaa

SEQ ID NO: 29 - DNA, 46 bp, Artificial Sequence
  Synthetic primers
cacacaggaaacagctatgaccatgtctgacataaaccaggccaac

SEQ ID NO: 30 - DNA, 44 bp, Artificial Sequence
  Synthetic primers
cacacaggaaacagctatgaccatgccgagtcctgggagttttg

SEQ ID NO: 31 - DNA, 45 bp, Artificial Sequence
  Synthetic primers
cacacaggaaacagctatgaccatgcgaggcactgcggtattaag

SEQ ID NO: 32 - DNA, 45 bp, Artificial Sequence
  Synthetic primers
cacacaggaaacagctatgaccatgacagccagtcgactctgagg

SEQ ID NO: 33 - DNA, 49 bp, Artificial Sequence
  Synthetic primers
cacacaggaaacagctatgaccatgaatggaacaaacaatgataagcaa

SEQ ID NO: 34 - DNA, 53 bp, Artificial Sequence; identical to SEQ ID NO: 14
  Synthetic primers

SEQ ID NO: 35 - DNA, 55 bp, Artificial Sequence
  Synthetic primers
cacacaggaaacagctatgaccatgactcacatgttgatttgacttactaatgta

SEQ ID NO: 36 - DNA, 52 bp, Artificial Sequence
  Synthetic primers
  misc_feature (1)...(52): n = A,T,C or G
cgacgtaaaacgacggccagtnnnnnnnnnnnnnngtgaggggccgtgttgt

SEQ ID NO: 37 - DNA, 57 bp, Artificial Sequence
  Synthetic primers
  misc_feature (1)...(57): n = A,T,C or G
cgacgtaaaacgacggccagtnnnnnnnnnnnnnncctgaattgtagcaatcaccaa

SEQ ID NO: 38 - DNA, 58 bp, Artificial Sequence
  Synthetic primers
  misc_feature (1)...(58): n = A,T,C or G
cgacgtaaaacgacggccagtnnnnnnnnnnnnnnccaccagtggaaataagaacaga

SEQ ID NO: 39 - DNA, 55 bp, Artificial Sequence
  Synthetic primers
  misc_feature (1)...(55): n = A,T,C or G
cgacgtaaaacgacggccagtnnnnnnnnnnnnnntccctcccctagaaggtctg

SEQ ID NO: 40 - DNA, 54 bp, Artificial Sequence
  Synthetic primers
  misc_feature (1)...(54): n = A,T,C or G
cgacgtaaaacgacggccagtnnnnnnnnnnnnnngcggtagcgatgaggtttc

SEQ ID NO: 41 - DNA, 56 bp, Artificial Sequence
  Synthetic primers
  misc_feature (1)...(56): n = A,T,C or G
cgacgtaaaacgacggccagtnnnnnnnnnnnnnnagagtcctttctcctgctgct

SEQ ID NO: 42 - DNA, 55 bp, Artificial Sequence
  Synthetic primers
  misc_feature (1)...(55): n = A,T,C or G
cgacgtaaaacgacggccagtnnnnnnnnnnnnnnttgcgtgtggagtatttgga

SEQ ID NO: 43 - DNA, 55 bp, Artificial Sequence
  Synthetic primers
  misc_feature (1)...(55): n = A,T,C or G
cgacgtaaaacgacggccagtnnnnnnnnnnnnnngttccccatttgaggtctcg

SEQ ID NO: 44 - DNA, 52 bp, Artificial Sequence
  Synthetic primers
  misc_feature (1)...(52): n = A,T,C or G
cgacgtaaaacgacggccagtnnnnnnnnnnnnnngcagcacgagggtcagg

SEQ ID NO: 45 - DNA, 55 bp, Artificial Sequence
  Synthetic primers
  misc_feature (1)...(55): n = A,T,C or G
cgacgtaaaacgacggccagtnnnnnnnnnnnnnntcattgggtgttacgcttcc

SEQ ID NO: 46 - DNA, 55 bp, Artificial Sequence
  Synthetic primers
  misc_feature (1)...(55): n = A,T,C or G
cgacgtaaaacgacggccagtnnnnnnnnnnnnnnagcaggcataggaacatcca

SEQ ID NO: 47 - DNA, 65 bp, Artificial Sequence
  Synthetic primers
  misc_feature (1)...(65): n = A,T,C or G
cgacgtaaaacgacggccagtnnnnnnnnnnnnnnatgcaaaatcacattattgccaacatgact

SEQ ID NO: 48 - DNA, 65 bp, Artificial Sequence; identical to SEQ ID NO: 47
  Synthetic primers
  misc_feature (1)...(65): n = A,T,C or G

SEQ ID NO: 49 - DNA, 55 bp, Artificial Sequence
  Synthetic primers
  misc_feature (1)...(55): n = A,T,C or G
cgacgtaaaacgacggccagtnnnnnnnnnnnnnntgtgatgatggtgaggatgg

SEQ ID NO: 50 - DNA, 50 bp, Artificial Sequence
  Synthetic primers
  misc_feature (1)...(50): n = A,T,C or G
cgacgtaaaacgacggccagtnnnnnnnnnnnnnncccgtcccgacccct

SEQ ID NO: 51 - DNA, 50 bp, Artificial Sequence; identical to SEQ ID NO: 50
  Synthetic primers
  misc_feature (1)...(50): n = A,T,C or G

SEQ ID NO: 52 - DNA, 53 bp, Artificial Sequence
  Synthetic primers
  misc_feature (1)...(53): n = A,T,C or G
cgacgtaaaacgacggccagtnnnnnnnnnnnnnngtggcaagtggctcctga

SEQ ID NO: 53 - DNA, 59 bp, Artificial Sequence
  Synthetic primers
  misc_feature (1)...(59): n = A,T,C or G
cgacgtaaaacgacggccagtnnnnnnnnnnnnnnaaagcccataaaggaatgtaaacc

SEQ ID NO: 54 - DNA, 53 bp, Artificial Sequence
  Synthetic primers
  misc_feature (1)...(53): n = A,T,C or G
cgacgtaaaacgacggccagtnnnnnnnnnnnnnncgggatggcttgaagaga

SEQ ID NO: 55 - DNA, 53 bp, Artificial Sequence
  Synthetic primers
  misc_feature (1)...(53): n = A,T,C or G
cgacgtaaaacgacggccagtnnnnnnnnnnnnnngggggtgtggaatcaacc

SEQ ID NO: 56 - DNA, 53 bp, Artificial Sequence
  Synthetic primers
  misc_feature (1)...(53): n = A,T,C or G
cgacgtaaaacgacggccagtnnnnnnnnnnnnnnggtggggagtgggactca

SEQ ID NO: 57 - DNA, 55 bp, Artificial Sequence
  Synthetic primers
  misc_feature (1)...(55): n = A,T,C or G
cgacgtaaaacgacggccagtnnnnnnnnnnnnnngttcagcctcctccctcatc

SEQ ID NO: 58 - DNA, 56 bp, Artificial Sequence
  Synthetic primers
  misc_feature (1)...(56): n = A,T,C or G
cgacgtaaaacgacggccagtnnnnnnnnnnnnnncatcagatacaacgccaccat

SEQ ID NO: 59 - DNA, 50 bp, Artificial Sequence; identical to SEQ ID NO: 50
  Synthetic primers
  misc_feature (1)...(50): n = A,T,C or G

SEQ ID NO: 60 - DNA, 50 bp, Artificial Sequence; identical to SEQ ID NO: 50
  Synthetic primers
  misc_feature (1)...(50): n = A,T,C or G

SEQ ID NO: 61 - DNA, 50 bp, Artificial Sequence; identical to SEQ ID NO: 50
  Synthetic primers
  misc_feature (1)...(50): n = A,T,C or G

SEQ ID NO: 62 - DNA, 50 bp, Artificial Sequence; identical to SEQ ID NO: 50
  Synthetic primers
  misc_feature (1)...(50): n = A,T,C or G

SEQ ID NO: 63 - DNA, 57 bp, Artificial Sequence
  Synthetic primers
  misc_feature (1)...(57): n = A,T,C or G
cgacgtaaaacgacggccagtnnnnnnnnnnnnnntggtccttacttccccatagaa

SEQ ID NO: 64 - DNA, 56 bp, Artificial Sequence
  Synthetic primers
  misc_feature (1)...(56): n = A,T,C or G
cgacgtaaaacgacggccagtnnnnnnnnnnnnnnaccaggtcttcgtaagcatga

SEQ ID NO: 65 - DNA, 55 bp, Artificial Sequence
  Synthetic primers
  misc_feature (1)...(55): n = A,T,C or G
cgacgtaaaacgacggccagtnnnnnnnnnnnnnntacagctgaggggaggagaa

SEQ ID NO: 66 - DNA, 55 bp, Artificial Sequence
  Synthetic primers
  misc_feature (1)...(55): n = A,T,C or G
cgacgtaaaacgacggccagtnnnnnnnnnnnnnntgggtcttcctcctcctctg

SEQ ID NO: 67 - DNA, 53 bp, Artificial Sequence
  Synthetic primers
  misc_feature (1)...(53): n = A,T,C or G
cgacgtaaaacgacggccagtnnnnnnnnnnnnnnatctgactccgccgattg

SEQ ID NO: 68 - DNA, 55 bp, Artificial Sequence
  Synthetic primers
  misc_feature (1)...(55): n = A,T,C or G
cgacgtaaaacgacggccagtnnnnnnnnnnnnnnggaaggggcgaaattacagt

SEQ ID NO: 69 - DNA, 55 bp, Artificial Sequence; identical to SEQ ID NO: 49
  Synthetic primers
  misc_feature (1)...(55): n = A,T,C or G

SEQ ID NO: 70 - DNA, 58 bp, Artificial Sequence
  Synthetic primers
  misc_feature (1)...(58): n = A,T,C or G
cgacgtaaaacgacggccagtnnnnnnnnnnnnnnacagtacaaaatggaggacctga